European Patent Specification EP 3 811 959 B1, published February 19, 2025. Title: COMPOSITION FOR PREVENTING OR TREATING MUSCLE DISEASE COMPRISING LICORICE EXTRACT OR COMPOUND ISOLATED THEREFROM AS ACTIVE INGREDIENT. Applicant: Research Cooperation Foundation of Yeungnam University Korea Institute of Oriental Medicine DAEGU CATHOLIC UNIVERSITY INDUSTRY ACADEMIC COOPERATION FOUNDATION. The sequence listing filed with the application follows.

SEQUENCE LISTING (14 sequences)

SEQ ID NO: 1 - DNA, 20 bp, Artificial Sequence
  GAPDH-f
tgctggtgctgagtatgtcg

SEQ ID NO: 2 - DNA, 20 bp, Artificial Sequence
  GAPDH-r
caagcagttggtggtacagg

SEQ ID NO: 3 - DNA, 20 bp, Artificial Sequence
  MYOD-f
aggagcacgcacacttctct

SEQ ID NO: 4 - DNA, 20 bp, Artificial Sequence
  MYOD-r
tctcgaaggcctcattcact

SEQ ID NO: 5 - DNA, 20 bp, Artificial Sequence
  MYOG-f
tccagtacattgagcgccta

SEQ ID NO: 6 - DNA, 20 bp, Artificial Sequence
  MYOG-r
caaatgatctcctgggttgg

SEQ ID NO: 7 - DNA, 20 bp, Artificial Sequence
  MYL2-f
aaagaggctccaggtccaat

SEQ ID NO: 8 - DNA, 20 bp, Artificial Sequence
  MYL2-r
cctctctgcttgtgtggtca

SEQ ID NO: 9 - DNA, 20 bp, Artificial Sequence
  Atrogin 1-f
ttcagcagcctgaactacga

SEQ ID NO: 10 - DNA, 20 bp, Artificial Sequence
  Atrogin 1-r
tgaaagcttcccccaaagta

SEQ ID NO: 11 - DNA, 20 bp, Artificial Sequence
  MuRf1-f
tgaggtgcctacttgctcct

SEQ ID NO: 12 - DNA, 20 bp, Artificial Sequence
  MuRf1-r
tcacctggtggctattctcc

SEQ ID NO: 13 - DNA, 20 bp, Artificial Sequence
  MSTN-f
acgctaccacggaaacaatc

SEQ ID NO: 14 - DNA, 20 bp, Artificial Sequence
  MSTN-r
ggagtcttgacgggtctgag